European Patent Application EP 4 779 314 A2, published July 22, 2026. Title: CONSTRUCT INCLUDING AN ANCHOR, AN ENZYME RECOGNITION SITE AND AN INDICATOR REGION FOR DETECTING MICROBIAL INFECTION IN WOUNDS. Applicant: SYNOVO GMBH. Application US 18/312,017, filed May 4, 2023. The sequence listing filed with the application follows.

SEQUENCE LISTING (46 sequences)

SEQ ID NO: 1-2 - skipped (2 entries)

SEQ ID NO: 3 - protein, 4 aa, synthetic construct
  REGION 1..4: note = Cathepsin G-specific substrate
AAPF

SEQ ID NO: 4 - protein, 4 aa, synthetic construct
  REGION 1..4: note = Cathepsin G-specific substrate
AAPM

SEQ ID NO: 5 - protein, 4 aa, synthetic construct
  REGION 1..4: note = Elastase substrate
AAPV

SEQ ID NO: 6 - protein, 5 aa, synthetic construct
  REGION 1..5: note = Protease substrate
APGGI

SEQ ID NO: 7 - protein, 4 aa, synthetic construct
  REGION 1..4: note = Protease substrate
MRRQ

SEQ ID NO: 8 - protein, 4 aa, synthetic construct
  REGION 1..4: note = Protease substrate
AAAA

SEQ ID NO: 9-10 - skipped (2 entries)

SEQ ID NO: 11 - protein, 5 aa, synthetic construct
  REGION 1..5: note = Protease substrate
  MOD_RES 1: note = the Xaa at position 1 is an alanine residue linked to an anchor moiety
XAAPV

SEQ ID NO: 12-17 - skipped (6 entries)

SEQ ID NO: 18 - protein, 6 aa, synthetic construct
  REGION 1..6: note = Protease substrate
  MOD_RES 1: note = the Xaa at position 1 is an alanine residue linked to an anchor moiety
  MOD_RES 6: note = the Xaa at position 6 is a valine residue linked to a moiety capable of causing a visible color change or a detectable electronic change, optionally via a linking moiety
XAPVAX

SEQ ID NO: 19 - protein, 5 aa, synthetic construct
  REGION 1..5: note = Protease substrate
  MOD_RES 1: note = the Xaa at position 1 is an alanine residue linked to an anchor moiety
XAPVA

SEQ ID NO: 20 - protein, 6 aa, synthetic construct
  REGION 1..6: note = Protease substrate
  MOD_RES 6: note = the Xaa at position 6 is a valine residue linked to a moiety capable of causing a visible color change or a detectable electronic change, optionally via a linking moiety
AAPVAX

SEQ ID NO: 21 - skipped

SEQ ID NO: 22 - protein, 6 aa, synthetic construct
  REGION 1..6: note = Protease substrate
  MOD_RES 1: note = the Xaa at position 1 is an alanine residue linked to an anchor moiety
  MOD_RES 6: note = the Xaa at position 6 is an alanine residue linked to a moiety capable of causing a visible color change or a detectable electronic change, optionally via a linking moiety
XAPVAX

SEQ ID NO: 23 - protein, 6 aa, synthetic construct
  REGION 1..6: note = Protease substrate
  MOD_RES 6: note = the Xaa at position 6 is an alanine residue linked to a moiety capable of causing a visible color change or a detectable electronic change, optionally via a linking moiety
AAPVAX

SEQ ID NO: 24 - skipped

SEQ ID NO: 25 - protein, 5 aa, synthetic construct
  REGION 1..5: note = Protease substrate
  MOD_RES 5: note = the Xaa at position 5 is an alanine residue linked to a moiety capable of causing a visible color change or a detectable electronic change, optionally via a linking moiety
AAPFX

SEQ ID NO: 26 - skipped

SEQ ID NO: 27 - protein, 5 aa, synthetic construct
  REGION 1..5: note = Protease substrate
  MOD_RES 1: note = the Xaa at position 1 is an alanine residue linked to an anchor moiety
XAPVA

SEQ ID NO: 28 - protein, 5 aa, synthetic construct
  REGION 1..5: note = Protease substrate
  MOD_RES 5: note = the Xaa at position 5 is an alanine residue linked to a moiety capable of causing a visible color change or a detectable electronic change, optionally via a linking moiety
AAPVX

SEQ ID NO: 29-32 - skipped (4 entries)

SEQ ID NO: 33 - protein, 5 aa, synthetic construct
  REGION 1..5: note = Protease substrate
  MOD_RES 5: note = the Xaa at position 5 is a methionine residue linked to a moiety capable of causing a visible color change or a detectable electronic change, optionally via a linking moiety
AAAPX

SEQ ID NO: 34 - protein, 5 aa, synthetic construct
  REGION 1..5: note = Protease substrate
  MOD_RES 5: note = the Xaa at position 5 is a valine residue linked to a moiety capable of causing a visible color change or a detectable electronic change, optionally via a linking moiety
AAAPX

SEQ ID NO: 35 - protein, 6 aa, synthetic construct
  REGION 1..6: note = Protease substrate
  MOD_RES 6: note = the Xaa at position 6 is a valine residue linked to a moiety capable of causing a visible color change or a detectable electronic change, optionally via a linking moiety
AAAPVX

SEQ ID NO: 36 - skipped

SEQ ID NO: 37 - protein, 6 aa, synthetic construct
  REGION 1..6: note = Protease substrate
  MOD_RES 1: note = the Xaa at position 1 is an alanine residue linked to an anchor moiety
  MOD_RES 6: note = the Xaa at position 6 is a valine residue linked to a moiety capable of causing a visible color change or a detectable electronic change, optionally via a linking moiety
XAAPVX

SEQ ID NO: 38 - protein, 6 aa, synthetic construct
  REGION 1..6: note = Protease substrate
  MOD_RES 1: note = the Xaa at position 1 is an alanine residue linked to an anchor moiety
XAAPVV

SEQ ID NO: 39 - protein, 4 aa, synthetic construct
  REGION 1..4: note = Protease substrate
AAPA

SEQ ID NO: 40 - protein, 6 aa, synthetic construct
  REGION 1..6: note = Consensus recognition motif for 3C protease
LEVLFQ

SEQ ID NO: 41 - protein, 4 aa, synthetic construct
  REGION 1..4: note = Consensus furin cleavage site
RRRR

SEQ ID NO: 42 - protein, 4 aa, synthetic construct
  REGION 1..4: note = Consensus furin cleavage site
RRKR

SEQ ID NO: 43 - protein, 4 aa, synthetic construct
  REGION 1..4: note = Consensus furin cleavage site
RLGR

SEQ ID NO: 44 - protein, 4 aa, synthetic construct
  REGION 1..4: note = Consensus furin cleavage site
LLGR

SEQ ID NO: 45 - protein, 4 aa, synthetic construct
  REGION 1..4: note = Consensus furin cleavage site
LLAR

SEQ ID NO: 46 - protein, 4 aa, synthetic construct
  REGION 1..4: note = Consensus furin cleavage site
LLAL